European Patent Application EP 4 786 003 A2, published August 5, 2026. Title: A FULLY NATIVE HUMAN NEUTRALIZING MONOCLONAL ANTIBODY AGAINST TETANUS TOXIN AND ITS APPLICATIONS. Applicant: ZHUHAI TRINOMAB BIOTECHNOLOGY CO., LTD. Application EP. The sequence listing filed with the application follows.

SEQUENCE LISTING (34 sequences)

SEQ ID NO: 1 - protein, 8 aa, synthetic construct
  REGION 1..8: note = antibody sequence
GGSISSYY

SEQ ID NO: 2 - protein, 7 aa, synthetic construct
  REGION 1..7: note = antibody sequence
VHYSGST

SEQ ID NO: 3 - protein, 12 aa, synthetic construct
  REGION 1..12: note = antibody sequence
ARDKYQTDVSDI

SEQ ID NO: 4 - protein, 7 aa, synthetic construct
  REGION 1..7: note = antibody sequence
QSITSSF

SEQ ID NO: 5 - skipped

SEQ ID NO: 6 - protein, 8 aa, synthetic construct
  REGION 1..8: note = antibody sequence
QQYDTSRT

SEQ ID NO: 7 - protein, 118 aa, synthetic construct
  REGION 1..118: note = antibody sequence
QVQLQESGPGLVKPSETLSLRCTVSGGSISSYYWSWFRQPPGKGLEWIGYVHYSGSTNYNPSLKSRFTLSVDTSKSQFSLRLRSVTAADTAIYYCARDKYQTDVSDIWGQGTVVTVSS

SEQ ID NO: 8 - protein, 107 aa, synthetic construct
  REGION 1..107: note = antibody sequence
DIQMTQSPGTLSLSPGERATLSCRASQSITSSFLAWYQQKPGQAPRLLIYGASSRATGIPDRFSGSGSGTDFILTISRLEPEDFAVYYCQQYDTSRTFGQGTTVEIK

SEQ ID NO: 9 - protein, 8 aa, synthetic construct
  REGION 1..8: note = antibody sequence
GYTFTNYW

SEQ ID NO: 10 - protein, 8 aa, synthetic construct
  REGION 1..8: note = antibody sequence
VYPGDSDT

SEQ ID NO: 11 - protein, 18 aa, synthetic construct
  REGION 1..18: note = antibody sequence
ATQQSNPYDSGSYWYFDS

SEQ ID NO: 12 - protein, 89 aa, synthetic construct
  REGION 1..89: note = antibody sequence
GYTFTNYWIGWVRQMPGKGLEWMGIVYPGDSDTRYSPSFQGQITISADKSISTAYLQWNNLKASDTGMYYCATQQSNPYDSGSYWYFDS

SEQ ID NO: 13 - protein, 6 aa, synthetic construct
  REGION 1..6: note = antibody sequence
QGIRNF

SEQ ID NO: 14 - skipped

SEQ ID NO: 15 - protein, 9 aa, synthetic construct
  REGION 1..9: note = antibody sequence
QKYFSAPPD

SEQ ID NO: 16 - protein, 71 aa, synthetic construct
  REGION 1..71: note = antibody sequence
QGIRNFLAWYQQKPGKVPKLLIYAASTLQSGVPSRFSGSGSGTDFTLTISSLQPEDVATYYCQKYFSAPPD

SEQ ID NO: 17 - protein, 125 aa, synthetic construct
  REGION 1..125: note = antibody sequence
EVQLVQSGAEVKKPGESLRISCQGSGYTFTNYWIGWVRQMPGKGLEWMGIVYPGDSDTRYSPSFQGQITISADKSISTAYLQWNNLKASDTGMYYCATQQSNPYDSGSYWYFDSWGQGTLVTVSS

SEQ ID NO: 18 - protein, 107 aa, synthetic construct
  REGION 1..107: note = antibody sequence
DIVMTQSPPSLSASIGDRVTITCRASQGIRNFLAWYQQKPGKVPKLLIYAASTLQSGVPSRFSGSGSGTDFTLTISSLQPEDVATYYCQKYFSAPPDFGQGTRLEIK

SEQ ID NO: 19 - protein, 8 aa, synthetic construct
  REGION 1..8: note = antibody sequence
GGPFTGSY

SEQ ID NO: 20 - protein, 7 aa, synthetic construct
  REGION 1..7: note = antibody sequence
VSQSGST

SEQ ID NO: 21 - protein, 12 aa, synthetic construct
ARLTKHYINSAY

SEQ ID NO: 22 - protein, 118 aa, synthetic construct
  REGION 1..118: note = antibody sequence
QVQLQESGAGLVKPSETLSLTCGVAGGPFTGSYLSWIRQPPGKGLEWIGEVSQSGSTSYNPSLKSRVTISVDTSKSQFSLKLSSVTAADTAVYYCARLTKHYINSAYWGQGTLVTVSS

SEQ ID NO: 23 - protein, 6 aa, synthetic construct
  REGION 1..6: note = antibody sequence
QIIGSW

SEQ ID NO: 24 - skipped

SEQ ID NO: 25 - protein, 9 aa, synthetic construct
  REGION 1..9: note = antibody sequence
QQYNSYPYT

SEQ ID NO: 26 - protein, 107 aa, synthetic construct
  REGION 1..107: note = antibody sequence
DIQMTQSPSILSASVGDRVTITCRASQIIGSWLAWYQQKPGKAPTLVIYKASRLDSGVPSRFSGTESGTEFTLTISSLQPDDFATYYCQQYNSYPYTFGQGTKLEIK

SEQ ID NO: 27 - protein, 8 aa, synthetic construct
  REGION 1..8: note = antibody sequence
GFGIGIYT

SEQ ID NO: 28 - protein, 8 aa, synthetic construct
  REGION 1..8: note = antibody sequence
ISGTSQYI

SEQ ID NO: 29 - protein, 8 aa, synthetic construct
  REGION 1..8: note = antibody sequence
VSGSSLDY

SEQ ID NO: 30 - protein, 6 aa, synthetic construct
  REGION 1..6: note = antibody sequence
QNIGTN

SEQ ID NO: 31 - skipped

SEQ ID NO: 32 - protein, 9 aa, synthetic construct
  REGION 1..9: note = antibody sequence
YQNYNSPKT

SEQ ID NO: 33 - protein, 115 aa, synthetic construct
  REGION 1..115: note = antibody sequence
EVQLVESGGGRVKPGGSLRLSCSVSGFGIGIYTMNWVRQAPGKGLEWVSSISGTSQYIYYANSVRGRFTISRDNAENSLYLQLNNLRAEDTALYYCVSGSSLDYWGQGTLVTISS

SEQ ID NO: 34 - protein, 107 aa, synthetic construct
  REGION 1..107: note = antibody sequence
DIQLTQSPSSLSASVGGRVTITCRASQNIGTNLNWFQQKPGTAPNLLIYGASTLQSGVPSRFSGSGSGTTFTLTIDSLQPEDFATYYCYQNYNSPKTFGQGTKVDLK